European Patent Application EP 4 265 613 A1, published October 25, 2023. Title: Benzene ring compound and use thereof. Applicant: NANJING SHIJIANG MEDICINE TECHNOLOGY CO., LTD. The sequence listing filed with the application follows.

SEQUENCE LISTING (1 sequence)

SEQ ID NO: 1 - DNA, 2500 bp, artificial sequence
  promoter region of NNMT gene
tatccaagagctatcagcactcccatgtttattgtagcactgttcacaatagccaagatttggaagtactctaagtgtccattagcagatgaatggataaagacaatgtggtaatacacataatggagtactattcagtcataaagaagaattagatcctgtcatttgcaataacatggatggaactggaggtcataatgttgagtgaaataaaccaggcacagaaagacaaactttgcatgttctcacttatttatgggagctaaaaactaaaataactgaactcacagagatagagagtagaaggatggttacgagaggatgggaagggtagcgaggtgggtaggggggatgtggggatcattaatgggtataaaaaatagttagaggccaggcgcagtggctcacgcctgtaatcccagcactttgggaggccgaggtaggcggaacacctgaggagttcaagaccagcctggccaatatgatgaaaccccgtctctactaaaaatacaaaaattagctgggcgtgatggtgtgcacctgtagtcccagctgcttgggaggctgaggcaggagaatcgctggaacccaagaggtgaaggttgcagtgagctgagatcgcgtcactgcactccagcctgggtgacagagtgagactccacatcaaaaaaaaaaaaaaaaagttagaaagattgaataagacctaatatttgctagcacaacagggtgaatatagtaaaaaataatttatttgtaccttcaaaaataactagacaagtataattgggttgtttgtaacacacaaaaaataagtacttgaagtggtggataccccatttaccctgatgtgattattttgtattgcaggcctctatcagaatatctcatgtaacccataaatatatacacctactctgtacccacaaaaagtttttaaaaagaaaaataaatagcaaccgaaaaaaaaagagagggagaaaagaaaaaagaaaaaaaaatcaagtgcctggctgggtagaataaattctaaggccacaatgttactgaccatgggttttttggctctcagtgtatagaaattgacacaaggccaatagtcttcccaaacatgctttactggaacttacgccctggcataagggccacaacaaaagagagagcgaattctctggcttgctgactccttggaaaaaaccggtagggatttttttattaggcaaagcacaggaattgacgtcagaggcaggatgtgctgctgggcaaagcatacgagaagtggggtatgcaggtcagcattacttggttgcaatggttatcttgaggaatgggccaactggtggtctggccagtggcaacaaggctgtaaatcaattattcagcattccttcccaaggtgggacacccggcaacattgtttatctcctaaggccagttcctggaattaagtgaaaggatgactaatggacatgttgtcagtgaggtagtggtgtgggttttgtgaccagtgggaatgcacgaaagaatgctttagcggggagtgagctgaagccaagccccatccctactctgtctcaaagtgagttcagaaaaggggatttaaagaattctttttttttttttttttttttttgagacagagtcttgctctgtcgcccaggctggagtgcagtggcgccatcttggctcactgcaagctccgccccccgggttcatgccattctcctgcctcagcctcccaagtagctgggactgcaggtgcctaccaccaagcccagctaattttttgtattttttttttagtagagacggggtttcaccatgttagccaggatggtctcgatctcctgacctcgtgatctgcccgccttagcctcccaaagtgctgggattacaggcatgagcctccgcccccggccttaaataattcttaaaggaagtaaagttaactttgaaagaactatcaggatttggattgactgaaaggagtggggaagcttagggaggaggtgcttgccagacactgggtcatggcagtggtcggtgaagctgcagttgcctagggcagggatggagagagagtctgggcatgaggagagggtctcgggatgtttggctggactagattttacagaaagccttatccaggcttttaaaattactctttccagacttcatctgagactccttcttcagccaacattccttagccctgaatacatttcctatcctcatctttcccttcttttttttcctttcttttacatgtttaaatttaaaccattcttcgtgaccccttttcttgggagattcatggcaagaacgagaagaatgatggtgcttgttaggggatgtcctgtctctctgaactttggggtcctatgcattaaataattttcctgacgagctcaagtgctccctctggtctacaatccctggcggctggccttcatcccttgggcaagcattgcatacagctcatggccctccctctaccataccc